European Patent Application EP 4 438 629 A1, published October 2, 2024. Title: MULTI-SPECIFIC LIGAND-BINDING MOLECULES AND APPLICATIONS THEREOF. Applicant: Suzhou light ferry Biomed. Co.,Ltd HK LIGHT FERRY BIOMED. LIMITED. The sequence listing filed with the application follows.

SEQUENCE LISTING (59 sequences)

SEQ ID NO: 1 - protein, 1338 aa, Homo sapiens
MVSYWDTGVLLCALLSCLLLTGSSSGSKLKDPELSLKGTQHIMQAGQTLHLQCRGEAAHKWSLPEMVSKESERLSITKSACGRNGKQFCSTLTLNTAQANHTGFYSCKYLAVPTSKKKETESAIYIFISDTGRPFVEMYSEIPEIIHMTEGRELVIPCRVTSPNITVTLKKFPLDTLIPDGKRIIWDSRKGFIISNATYKEIGLLTCEATVNGHLYKTNYLTHRQTNTIIDVQISTPRPVKLLRGHTLVLNCTATTPLNTRVQMTWSYPDEKNKRASVRRRIDQSNSHANIFYSVLTIDKMQNKDKGLYTCRVRSGPSFKSVNTSVHIYDKAFITVKHRKQQVLETVAGKRSYRLSMKVKAFPSPEVVWLKDGLPATEKSARYLTRGYSLIIKDVTEEDAGNYTILLSIKQSNVFKNLTATLIVNVKPQIYEKAVSSFPDPALYPLGSRQILTCTAYGIPQPTIKWFWHPCNHNHSEARCDFCSNNEESFILDADSNMGNRIESITQRMAIIEGKNKMASTLVVADSRISGIYICIASNKVGTVGRNISFYITDVPNGFHVNLEKMPTEGEDLKLSCTVNKFLYRDVTWILLRTVNNRTMHYSISKQKMAITKEHSITLNLTIMNVSLQDSGTYACRARNVYTGEEILQKKEITIRDQEAPYLLRNLSDHTVAISSSTTLDCHANGVPEPQITWFKNNHKIQQEPGIILGPGSSTLFIERVTEEDEGVYHCKATNQKGSVESSAYLTVQGTSDKSNLELITLTCTCVAATLFWLLLTLFIRKMKRSSSEIKTDYLSIIMDPDEVPLDEQCERLPYDASKWEFARERLKLGKSLGRGAFGKVVQASAFGIKKSPTCRTVAVKMLKEGATASEYKALMTELKILTHIGHHLNVVNLLGACTKQGGPLMVIVEYCKYGNLSNYLKSKRDLFFLNKDAALHMEPKKEKMEPGLEQGKKPRLDSVTSSESFASSGFQEDKSLSDVEEEEDSDGFYKEPITMEDLISYSFQVARGMEFLSSRKCIHRDLAARNILLSENNVVKICDFGLARDIYKNPDYVRKGDTRLPLKWMAPESIFDKIYSTKSDVWSYGVLLWEIFSLGGSPYPGVQMDEDFCSRLREGMRMRAPEYSTPEIYQIMLDCWHRDPKERPRFAELVEKLGDLLQANVQQDGKDYIPINAILTGNSGFTYSTPAFSEDFFKESISAPKFNSGSSDDVRYVNAFKFMSLERIKTFEELLPNATSMFDDYQGDSSTLLASPMLKRFTWTDSKPKASLKIDLRVTSKSKESGLSDVSRPSFCHSSCGHVSEGKRRFTYDHAELERKIACCSPPPDYNSVVLYSTPPI

SEQ ID NO: 2 - protein, 1356 aa, Homo sapiens
MQSKVLLAVALWLCVETRAASVGLPSVSLDLPRLSIQKDILTIKANTTLQITCRGQRDLDWLWPNNQSGSEQRVEVTECSDGLFCKTLTIPKVIGNDTGAYKCFYRETDLASVIYVYVQDYRSPFIASVSDQHGVVYITENKNKTVVIPCLGSISNLNVSLCARYPEKRFVPDGNRISWDSKKGFTIPSYMISYAGMVFCEAKINDESYQSIMYIVVVVGYRIYDVVLSPSHGIELSVGEKLVLNCTARTELNVGIDFNWEYPSSKHQHKKLVNRDLKTQSGSEMKKFLSTLTIDGVTRSDQGLYTCAASSGLMTKKNSTFVRVHEKPFVAFGSGMESLVEATVGERVRIPAKYLGYPPPEIKWYKNGIPLESNHTIKAGHVLTIMEVSERDTGNYTVILTNPISKEKQSHVVSLVVYVPPQIGEKSLISPVDSYQYGTTQTLTCTVYAIPPPHHIHWYWQLEEECANEPSQAVSVTNPYPCEEWRSVEDFQGGNKIEVNKNQFALIEGKNKTVSTLVIQAANVSALYKCEAVNKVGRGERVISFHVTRGPEITLQPDMQPTEQESVSLWCTADRSTFENLTWYKLGPQPLPIHVGELPTPVCKNLDTLWKLNATMFSNSTNDILIMELKNASLQDQGDYVCLAQDRKTKKRHCVVRQLTVLERVAPTITGNLENQTTSIGESIEVSCTASGNPPPQIMWFKDNETLVEDSGIVLKDGNRNLTIRRVRKEDEGLYTCQACSVLGCAKVEAFFIIEGAQEKTNLEIIILVGTAVIAMFFWLLLVIILRTVKRANGGELKTGYLSIVMDPDELPLDEHCERLPYDASKWEFPRDRLKLGKPLGRGAFGQVIEADAFGIDKTATCRTVAVKMLKEGATHSEHRALMSELKILIHIGHHLNVVNLLGACTKPGGPLMVIVEFCKFGNLSTYLRSKRNEFVPYKTKGARFRQGKDYVGAIPVDLKRRLDSITSSQSSASSGFVEEKSLSDVEEEEAPEDLYKDFLTLEHLICYSFQVAKGMEFLASRKCIHRDLAARNILLSEKNVVKICDFGLARDIYKDPDYVRKGDARLPLKWMAPETIFDRVYTIQSDVWSFGVLLWEIFSLGASPYPGVKIDEEFCRRLKEGTRMRAPDYTTPEMYQTMLDCWHGEPSQRPTFSELVEHLGNLLQANAQQDGKDYIVLPISETLSMEEDSGLSLPTSPVSCMEEEEVCDPKFHYDNTAGISQYLQNSKRKSRPVSVKTFEDIPLEEPEVKVIPDDNQTDSGMVLASEELKTLEDRTKLSPSFGGMVPSKSRESVASEGSNQTSGYQSGYHSDDTDTTVYSSEEAELLKLIEIGVQTGSTAQILQPDSGTTLSSPPV

SEQ ID NO: 3 - protein, 1363 aa, Homo sapiens
MQRGAALCLRLWLCLGLLDGLVSGYSMTPPTLNITEESHVIDTGDSLSISCRGQHPLEWAWPGAQEAPATGDKDSEDTGVVRDCEGTDARPYCKVLLLHEVHANDTGSYVCYYKYIKARIEGTTAASSYVFVRDFEQPFINKPDTLLVNRKDAMWVPCLVSIPGLNVTLRSQSSVLWPDGQEVVWDDRRGMLVSTPLLHDALYLQCETTWGDQDFLSNPFLVHITGNELYDIQLLPRKSLELLVGEKLVLNCTVWAEFNSGVTFDWDYPGKQAERGKWVPERRSQQTHTELSSILTIHNVSQHDLGSYVCKANNGIQRFRESTEVIVHENPFISVEWLKGPILEATAGDELVKLPVKLAAYPPPEFQWYKDGKALSGRHSPHALVLKEVTEASTGTYTLALWNSAAGLRRNISLELVVNVPPQIHEKEASSPSIYSRHSRQALTCTAYGVPLPLSIQWHWRPWTPCKMFAQRSLRRRQQQDLMPQCRDWRAVTTQDAVNPIESLDTWTEFVEGKNKTVSKLVIQNANVSAMYKCVVSNKVGQDERLIYFYVTTIPDGFTIESKPSEELLEGQPVLLSCQADSYKYEHLRWYRLNLSTLHDAHGNPLLLDCKNVHLFATPLAASLEEVAPGARHATLSLSIPRVAPEHEGHYVCEVQDRRSHDKHCHKKYLSVQALEAPRLTQNLTDLLVNVSDSLEMQCLVAGAHAPSIVWYKDERLLEEKSGVDLADSNQKLSIQRVREEDAGRYLCSVCNAKGCVNSSASVAVEGSEDKGSMEIVILVGTGVIAVFFWVLLLLIFCNMRRPAHADIKTGYLSIIMDPGEVPLEEQCEYLSYDASQWEFPRERLHLGRVLGYGAFGKVVEASAFGIHKGSSCDTVAVKMLKEGATASEHRALMSELKILIHIGNHLNVVNLLGACTKPQGPLMVIVEFCKYGNLSNFLRAKRDAFSPCAEKSPEQRGRFRAMVELARLDRRRPGSSDRVLFARFSKTEGGARRASPDQEAEDLWLSPLTMEDLVCYSFQVARGMEFLASRKCIHRDLAARNILLSESDVVKICDFGLARDIYKDPDYVRKGSARLPLKWMAPESIFDKVYTTQSDVWSFGVLLWEIFSLGASPYPGVQINEEFCQRLRDGTRMRAPELATPAIRRIMLNCWSGDPKARPAFSELVEILGDLLQGRGLQEEEEVCMAPRSSQSSEEGSFSQVSTMALHIAQADAEDSPPSLQRHSLAARYYNWVSFPGCLARGAETRGSSRMKTFEEFPMTPTTYKGSVDNQTDSGMVLASEEFEQIESRHRQESGFSCKGPGQNVAVTRAHPDSQGRRRRPERGARGGQVFYNSEYGELSEPSEEDHCSPSARVTFFTDNSY

SEQ ID NO: 4 - protein, 102 aa, Artificial sequence
  LFV-A Trap polypeptide
YVQDYRSPFIASVSDQHGVVYITENKNKTVVIPCLGSISNLNVSLCARYPEKRFVPDGNRISWDSKKGFTIPSYMISYAGMVFCEAKINDESYQSIMYIVVV

SEQ ID NO: 5 - protein, 211 aa, Artificial sequence
  LFV-B Trap polypeptide
YVQDYRSPFIASVSDQHGVVYITENKNKTVVIPCLGSISNLNVSLCARYPEKRFVPDGNRISWDSKKGFTIPSYMISYAGMVFCEAKINDESYQSIMYIVVVVGYRIYDVVLSPSHGIELSVGEKLVLNCTARTELNVGIDFNWEYPSSKHQHKKLVNRDLKTQSGSEMKKFLSTLTIDGVTRSDQGLYTCAASSGLMTKKNSTFVRVHEK

SEQ ID NO: 6 - protein, 205 aa, Artificial sequence
  LFV-C Trap polypeptide
SPFIASVSDQHGVVYITENKNKTVVIPCLGSISNLNVSLCARYPEKRFVPDGNRISWDSKKGFTIPSYMISYAGMVFCEAKINDESYQSIMYIVVVVGYRIYDVVLSPSHGIELSVGEKLVLNCTARTELNVGIDFNWEYPSSKHQHKKLVNRDLKTQSGSEMKKFLSTLTIDGVTRSDQGLYTCAASSGLMTKKNSTFVRVHEK

SEQ ID NO: 7 - protein, 305 aa, Artificial sequence
  LFV-D Trap polypeptide
YVQDYRSPFIASVSDQHGVVYITENKNKTVVIPCLGSISNLNVSLCARYPEKRFVPDGNRISWDSKKGFTIPSYMISYAGMVFCEAKINDESYQSIMYIVVVVGYRIYDVVLSPSHGIELSVGEKLVLNCTARTELNVGIDFNWEYPSSKHQHKKLVNRDLKTQSGSEMKKFLSTLTIDGVTRSDQGLYTCAASSGLMTKKNSTFVRVHEKPFVAFGSGMESLVEATVGERVRIPAKYLGYPPPEIKWYKNGIPLESNHTIKAGHVLTIMEVSERDTGNYTVILTNPISKEKQSHVVSLVVYVPP

SEQ ID NO: 8 - protein, 305 aa, Artificial sequence
  LFV-E Trap polypeptide
GLPSVSLDLPRLSIQKDILTIKANTTLQITCRGQRDLDWLWPNNQSGSEQRVEVTECSDGLFCKTLTIPKVIGNDTGAYKCFYRETDLASVIYVYVQDYRSPFIASVSDQHGVVYITENKNKTVVIPCLGSISNLNVSLCARYPEKRFVPDGNRISWDSKKGFTIPSYMISYAGMVFCEAKINDESYQSIMYIVVVVGYRIYDVVLSPSHGIELSVGEKLVLNCTARTELNVGIDFNWEYPSSKHQHKKLVNRDLKTQSGSEMKKFLSTLTIDGVTRSDQGLYTCAASSGLMTKKNSTFVRVHEK

SEQ ID NO: 9 - protein, 399 aa, Artificial sequence
  LFV-F Trap polypeptide
GLPSVSLDLPRLSIQKDILTIKANTTLQITCRGQRDLDWLWPNNQSGSEQRVEVTECSDGLFCKTLTIPKVIGNDTGAYKCFYRETDLASVIYVYVQDYRSPFIASVSDQHGVVYITENKNKTVVIPCLGSISNLNVSLCARYPEKRFVPDGNRISWDSKKGFTIPSYMISYAGMVFCEAKINDESYQSIMYIVVVVGYRIYDVVLSPSHGIELSVGEKLVLNCTARTELNVGIDFNWEYPSSKHQHKKLVNRDLKTQSGSEMKKFLSTLTIDGVTRSDQGLYTCAASSGLMTKKNSTFVRVHEKPFVAFGSGMESLVEATVGERVRIPAKYLGYPPPEIKWYKNGIPLESNHTIKAGHVLTIMEVSERDTGNYTVILTNPISKEKQSHVVSLVVYVPP

SEQ ID NO: 10 - protein, 205 aa, Artificial sequence
  LFV-G Trap polypeptide
SPFIASVSDQHGVVYITENKAKTVVIPCLGSISNLNVSLCARYPEKRFVPDGNRISWDSKKGFTIPSYMISYAGMVFCEAKINDESYQSIMYIVVVVGYRIYDVVLSPSHGIELSVGEKLVLNCTARTELNVGIDFNWEYPSSKHQHKKLVNRDLKTQSGSEMKKFLSTLTIDGVTRSDQGLYTCAASSGLMTKKNSTFVRVHEK

SEQ ID NO: 11 - protein, 205 aa, Artificial sequence
  LFV-H Trap polypeptide
SPFIASVSDQHGVVYITENKQKTVVIPCLGSISNLNVSLCARYPEKRFVPDGNRISWDSKKGFTIPSYMISYAGMVFCEAKINDESYQSIMYIVVVVGYRIYDVVLSPSHGIELSVGEKLVLNCTARTELNVGIDFNWEYPSSKHQHKKLVNRDLKTQSGSEMKKFLSTLTIDGVTRSDQGLYTCAASSGLMTKKNSTFVRVHEK

SEQ ID NO: 12 - protein, 205 aa, Artificial sequence
  LFV-I Trap polypeptide
SPFIASVSDQHGVVYITENKNKTVVIPCLGSISNLAVSLCARYPEKRFVPDGNRISWDSKKGFTIPSYMISYAGMVFCEAKINDESYQSIMYIVVVVGYRIYDVVLSPSHGIELSVGEKLVLNCTARTELNVGIDFNWEYPSSKHQHKKLVNRDLKTQSGSEMKKFLSTLTIDGVTRSDQGLYTCAASSGLMTKKNSTFVRVHEK

SEQ ID NO: 13 - protein, 205 aa, Artificial sequence
  LFV-J Trap polypeptide
SPFIASVSDQHGVVYITENKNKTVVIPCLGSISNLQVSLCARYPEKRFVPDGNRISWDSKKGFTIPSYMISYAGMVFCEAKINDESYQSIMYIVVVVGYRIYDVVLSPSHGIELSVGEKLVLNCTARTELNVGIDFNWEYPSSKHQHKKLVNRDLKTQSGSEMKKFLSTLTIDGVTRSDQGLYTCAASSGLMTKKNSTFVRVHEK

SEQ ID NO: 14 - protein, 205 aa, Artificial sequence
  LFV-K Trap polypeptide
SPFIASVSDQHGVVYITENKNKTVVIPCLGSISNLNVSLCARYPEKRFVPDGNRISWDSKKGFTIPSYMISYAGMVFCEAKINDESYQSIMYIVVVVGYRIYDVVLSPSHGIELSVGEKLVLQCTARTELNVGIDFNWEYPSSKHQHKKLVNRDLKTQSGSEMKKFLSTLTIDGVTRSDQGLYTCAASSGLMTKKNSTFVRVHEK

SEQ ID NO: 15 - protein, 205 aa, Artificial sequence
  LFV-L Trap polypeptide
SPFIASVSDQHGVVYITENKNKTVVIPCLGSISNLNVSLCARYPEKRFVPDGNRISWDSKKGFTIPSYMISYAGMVFCEAKINDESYQSIMYIVVVVGYRIYDVVLSPSHGIELSVGEKLVLNCTARTELNVGIDFNWEYPSSKHQHKKLVNRDLKTQSGSEMKKFLSTLTIDGVTRSDQGLYTCAASSGLMTKKQSTFVRVHEK

SEQ ID NO: 16 - protein, 311 aa, Artificial sequence
  LFV-M Trap polypeptide
GRPFVEMYSEIPEIIHMTEGRELVIPCRVTSPNITVTLKKFPLDTLIPDGKRIIWDSRKGFIISNATYKEIGLLTCEATVNGHLYKTNYLTHRQTNTIIGGGGSGGSPFIASVSDQHGVVYITENKNKTVVIPCLGSISNLNVSLCARYPEKRFVPDGNRISWDSKKGFTIPSYMISYAGMVFCEAKINDESYQSIMYIVVVVGYRIYDVVLSPSHGIELSVGEKLVLNCTARTELNVGIDFNWEYPSSKHQHKKLVNRDLKTQSGSEMKKFLSTLTIDGVTRSDQGLYTCAASSGLMTKKNSTFVRVHEK

SEQ ID NO: 17 - protein, 309 aa, Artificial sequence
  LFV-N Trap polypeptide
SPFIASVSDQHGVVYITENKNKTVVIPCLGSISNLNVSLCARYPEKRFVPDGNRISWDSKKGFTIPSYMISYAGMVFCEAKINDESYQSIMYIVVVVGYRIYDVVLSPSHGIELSVGEKLVLNCTARTELNVGIDFNWEYPSSKHQHKKLVNRDLKTQSGSEMKKFLSTLTIDGVTRSDQGLYTCAASSGLMTKKNSTFVRVHEKGGGGSGRPFVEMYSEIPEIIHMTEGRELVIPCRVTSPNITVTLKKFPLDTLIPDGKRIIWDSRKGFIISNATYKEIGLLTCEATVNGHLYKTNYLTHRQTNTII

SEQ ID NO: 18 - protein, 211 aa, Artificial sequence
  LFV-P Trap polypeptide
YVQDYRSPFIASVSDQHGVVYITENKNKTVVIPCLGSISNLNVSLCARYPEKRFVPDGNRISWDSKKGFTIPSYMISYAGMVFCEAKINDESYQSIMYIVVVVGYRIYDVVLSPSHGIELSVGEKLVLQCTARTELNVGIDFNWEYPSSKHQHKKLVNRDLKTQSGSEMKKFLSTLTIDGVTRSDQGLYTCAASSGLMTKKNSTFVRVHEK

SEQ ID NO: 19 - protein, 315 aa, Artificial sequence
  LFV-Q Trap polypeptide
YVQDYRSPFIASVSDQHGVVYITENKNKTVVIPCLGSISNLNVSLCARYPEKRFVPDGNRISWDSKKGFTIPSYMISYAGMVFCEAKINDESYQSIMYIVVVVGYRIYDVVLSPSHGIELSVGEKLVLQCTARTELNVGIDFNWEYPSSKHQHKKLVNRDLKTQSGSEMKKFLSTLTIDGVTRSDQGLYTCAASSGLMTKKNSTFVRVHEKGGGGSGRPFVEMYSEIPEIIHMTEGRELVIPCRVTSPNITVTLKKFPLDTLIPDGKRIIWDSRKGFIISNATYKEIGLLTCEATVNGHLYKTNYLTHRQTNTII

SEQ ID NO: 20 - protein, 311 aa, Artificial sequence
  LFV-R Trap polypeptide
GRPFVEMYSEIPEIIHMTEGRELVIPCRVTSPNITVTLKKFPLDTLIPDGKRIIWDSRKGFIISNATYKEIGLLTCEATVNGHLYKTNYLTHRQTNTIIGGGGSGGSPFIASVSDQHGVVYITENKNKTVVIPCLGSISNLNVSLCARYPEKRFVPDGNRISWDSKKGFTIPSYMISYAGMVFCEAKINDESYQSIMYIVVVVGYRIYDVVLSPSHGIELSVGEKLVLQCTARTELNVGIDFNWEYPSSKHQHKKLVNRDLKTQSGSEMKKFLSTLTIDGVTRSDQGLYTCAASSGLMTKKNSTFVRVHEK

SEQ ID NO: 21 - protein, 315 aa, Artificial sequence
  LFV-S Trap polypeptide
YVQDYRSPFIASVSDQHGVVYITENKNKTVVIPCLGSISNLNVSLCARYPEKRFVPDGNRISWDSKKGFTIPSYMISYAGMVFCEAKINDESYQSIMYIVVVVGYRIYDVVLSPSHGIELSVGEKLVLNCTARTELNVGIDFNWEYPSSKHQHKKLVNRDLKTQSGSEMKKFLSTLTIDGVTRSDQGLYTCAASSGLMTKKNSTFVRVHEKGGGGSGRPFVEMYSEIPEIIHMTEGRELVIPCRVTSPNITVTLKKFPLDTLIPDGKRIIWDSRKGFIISNATYKEIGLLTCEATVNGHLYKTNYLTHRQTNTII

SEQ ID NO: 22 - protein, 309 aa, Artificial sequence
  LFV-001 Trap polypeptide
YSMTPPTLNITEESHVIDTGDSLSISCRGQHPLEWAWPGAQEAPATGDKDSEDTGVVRDCEGTDARPYCKVLLLHEVHANDTGSYVCYYKYIKARIEGTTAASSYVFVRDFEQPFINKPDTLLVNRKDAMWVPCLVSIPGLNVTLRSQSSVLWPDGQEVVWDDRRGMLVSTPLLHDALYLQCETTWGDQDFLSNPFLVHITGYRIYDVVLSPSHGIELSVGEKLVLNCTARTELNVGIDFNWEYPSSKHQHKKLVNRDLKTQSGSEMKKFLSTLTIDGVTRSDQGLYTCAASSGLMTKKNSTFVRVHEK

SEQ ID NO: 23 - protein, 309 aa, Artificial sequence
  LFV-010 Trap polypeptide
YSMTPPTLNITEESHVIDTGDSLSISCRGQHPLEWAWPGAQEAPATGDKDSEDTGVVRDCEGTDARPYCKVLLLHEVHAQDTGSYVCYYKYIKARIEGTTAASSYVFVRDFEQPFINKPDTLLVNRKDAMWVPCLVSIPGLNVTLRSQSSVLWPDGQEVVWDDRRGMLVSTPLLHDALYLQCETTWGDQDFLSNPFLVHITGNELYDVVLSPSHGIELSVGEKLVLNCTARTELNVGIDFNWEYPSSKHQHKKLVNRDLKTQSGSEMKKFLSTLTIDGVTRSDQGLYTCAASSGLMTKKNSTFVRVHEK

SEQ ID NO: 24 - protein, 308 aa, Artificial sequence
  LFV-002 Trap polypeptide
YSMTPPTLNITEESHVIDTGDSLSISCRGQHPLEWAWPGAQEAPATGDKDSEDTGVVRDCEGTDARPYCKVLLLHEVHANDTGSYVCYYKYIKARIEGTTAASSYVFVRDFEQPFINKPDTLLVNRKDAMWVPCLVSIPGLNVTLRSQSSVLWPDGQEVVWDDRRGMLVSTPLLHDALYLQCETTWGDQDFLSNPFLVHIGYRIYDVVLSPSHGIELSVGEKLVLNCTARTELNVGIDFNWEYPSSKHQHKKLVNRDLKTQSGSEMKKFLSTLTIDGVTRSDQGLYTCAASSGLMTKKNSTFVRVHEK

SEQ ID NO: 25 - protein, 309 aa, Artificial sequence
  LFV-003 Trap polypeptide
YSMTPPTLNITEESHVIDTGDSLSISCRGQHPLEWAWPGAQEAPATGDKDSEDTGVVRDCEGTDARPYCKVLLLHEVHANDTGSYVCYYKYIKARIEGTTAASSYVFVRDFEQPFINKPDTLLVNRKDAMWVPCLVSIPGLNVTLRSQSSVLWPDGQEVVWDDRRGMLVSTPLLHDALYLQCETTWGDQDFLSNPFLVHIGGYRIYDVVLSPSHGIELSVGEKLVLNCTARTELNVGIDFNWEYPSSKHQHKKLVNRDLKTQSGSEMKKFLSTLTIDGVTRSDQGLYTCAASSGLMTKKNSTFVRVHEK

SEQ ID NO: 26 - protein, 309 aa, Artificial sequence
  LFV-004 Trap polypeptide
YSMTPPTLNITEESHVIDTGDSLSISCRGQHPLEWAWPGAQEAPATGDKDSEDTGVVRDCEGTDARPYCKVLLLHEVHANDTGSYVCYYKYIKARIEGTTAASSYVFVRDFEQPFINKPDTLLVNRKDAMWVPCLVSIPGLNVTLRSQSSVLWPDGQEVVWDDRRGMLVSTPLLHDALYLQCETTWGDQDFLSNPFIVHVTGYRIYDVVLSPSHGIELSVGEKLVLNCTARTELNVGIDFNWEYPSSKHQHKKLVNRDLKTQSGSEMKKFLSTLTIDGVTRSDQGLYTCAASSGLMTKKNSTFVRVHEK

SEQ ID NO: 27 - protein, 309 aa, Artificial sequence
  LFV-005 Trap polypeptide
YSMTPPTLNITEESHVIDTGDSLSISCRGQHPLEWAWPGAQEAPATGDKDSEDTGVVRDCEGTDARPYCKVLLLHEVHANDTGSYVCYYKYIKARIEGTTAASSYVFVRDFEQPFINKPDTLLVNRKDAMWVPCLVSIPGLNVTLRSQSSVLWPDGQEVVWDDRRGMLVSTPLLHDALYLQCETTWGDQDFLSNPFIVVVVGYRIYDVVLSPSHGIELSVGEKLVLNCTARTELNVGIDFNWEYPSSKHQHKKLVNRDLKTQSGSEMKKFLSTLTIDGVTRSDQGLYTCAASSGLMTKKNSTFVRVHEK

SEQ ID NO: 28 - protein, 309 aa, Artificial sequence
  LFV-006 Trap polypeptide
YSMTPPTLNITEESHVIDTGDSLSISCRGQHPLEWAWPGAQEAPATGDKDSEDTGVVRDCEGTDARPYCKVLLLHEVHANDTGSYVCYYKYIKARIEGTTAASSYVFVRDFEQPFINKPDTLLVNRKDAMWVPCLVSIPGLNVTLRSQSSVLWPDGQEVVWDDRRGMLVSTPLLHDALYLQCETTWGDQDFLSNMYIVVVVGYRIYDVVLSPSHGIELSVGEKLVLNCTARTELNVGIDFNWEYPSSKHQHKKLVNRDLKTQSGSEMKKFLSTLTIDGVTRSDQGLYTCAASSGLMTKKNSTFVRVHEK

SEQ ID NO: 29 - protein, 309 aa, Artificial sequence
  LFV-007 Trap polypeptide
YSMTPPTLNITEESHVIDTGDSLSISCRGQHPLEWAWPGAQEAPATGDKDSEDTGVVRDCEGTDARPYCKVLLLHEVHANDTGSYVCYYKYIKARIEGTTAASSYVFVRDFEQPFINKPDTLLVNRKDAMWVPCLVSIPGLNVTLRSQSSVLWPDGQEVVWDDRRGMLVSTPLLHDALYLQCETTWGDQDFLSIMYIVVVVGYRIYDVVLSPSHGIELSVGEKLVLNCTARTELNVGIDFNWEYPSSKHQHKKLVNRDLKTQSGSEMKKFLSTLTIDGVTRSDQGLYTCAASSGLMTKKNSTFVRVHEK

SEQ ID NO: 30 - protein, 309 aa, Artificial sequence
  LFV-008 Trap polypeptide
YSMTPPTLNITEESHVIDTGDSLSISCRGQHPLEWAWPGAQEAPATGDKDSEDTGVVRDCEGTDARPYCKVLLLHEVHANDTGSYVCYYKYIKARIEGTTAASSYVFVRDFEQPFINKPDTLLVNRKDAMWVPCLVSIPGLNVTLRSQSSVLWPDGQEVVWDDRRGMLVSTPLLHDALYLQCETTWGDQDFLSAMYIVVVVGYRIYDVVLSPSHGIELSVGEKLVLNCTARTELNVGIDFNWEYPSSKHQHKKLVNRDLKTQSGSEMKKFLSTLTIDGVTRSDQGLYTCAASSGLMTKKNSTFVRVHEK

SEQ ID NO: 31 - protein, 330 aa, Homo sapiens [sequence omitted]

SEQ ID NO: 32 - protein, 332 aa, Artificial sequence
  LFV-A recombinant receptor molecule
YVQDYRSPFIASVSDQHGVVYITENKNKTVVIPCLGSISNLNVSLCARYPEKRFVPDGNRISWDSKKGFTIPSYMISYAGMVFCEAKINDESYQSIMYIVVVGPGDKTHTCPPCPAPELLGGPSVFLFPPKPKDTLMISRTPEVTCVVVDVSHEDPEVKFNWYVDGVEVHNAKTKPREEQYNSTYRVVSVLTVLHQDWLNGKEYKCKVSNKALPAPIEKTISKAKGQPREPQVYTLPPSRDELTKNQVSLTCLVKGFYPSDIAVEWESNGQPENNYKTTPPVLDSDGSFFLYSKLTVDKSRWQQGNVFSCSVMHEALHNHYTQKSLSLSPGK

SEQ ID NO: 33 - protein, 441 aa, Artificial sequence
  LFV-B recombinant receptor molecule
YVQDYRSPFIASVSDQHGVVYITENKNKTVVIPCLGSISNLNVSLCARYPEKRFVPDGNRISWDSKKGFTIPSYMISYAGMVFCEAKINDESYQSIMYIVVVVGYRIYDVVLSPSHGIELSVGEKLVLNCTARTELNVGIDFNWEYPSSKHQHKKLVNRDLKTQSGSEMKKFLSTLTIDGVTRSDQGLYTCAASSGLMTKKNSTFVRVHEKGPGDKTHTCPPCPAPELLGGPSVFLFPPKPKDTLMISRTPEVTCVVVDVSHEDPEVKFNWYVDGVEVHNAKTKPREEQYNSTYRVVSVLTVLHQDWLNGKEYKCKVSNKALPAPIEKTISKAKGQPREPQVYTLPPSRDELTKNQVSLTCLVKGFYPSDIAVEWESNGQPENNYKTTPPVLDSDGSFFLYSKLTVDKSRWQQGNVFSCSVMHEALHNHYTQKSLSLSPGK

SEQ ID NO: 34 - protein, 435 aa, Artificial sequence
  LFV-C recombinant receptor molecule
SPFIASVSDQHGVVYITENKNKTVVIPCLGSISNLNVSLCARYPEKRFVPDGNRISWDSKKGFTIPSYMISYAGMVFCEAKINDESYQSIMYIVVVVGYRIYDVVLSPSHGIELSVGEKLVLNCTARTELNVGIDFNWEYPSSKHQHKKLVNRDLKTQSGSEMKKFLSTLTIDGVTRSDQGLYTCAASSGLMTKKNSTFVRVHEKGPGDKTHTCPPCPAPELLGGPSVFLFPPKPKDTLMISRTPEVTCVVVDVSHEDPEVKFNWYVDGVEVHNAKTKPREEQYNSTYRVVSVLTVLHQDWLNGKEYKCKVSNKALPAPIEKTISKAKGQPREPQVYTLPPSRDELTKNQVSLTCLVKGFYPSDIAVEWESNGQPENNYKTTPPVLDSDGSFFLYSKLTVDKSRWQQGNVFSCSVMHEALHNHYTQKSLSLSPGK

SEQ ID NO: 35 - protein, 535 aa, Artificial sequence
  LFV-D recombinant receptor molecule
YVQDYRSPFIASVSDQHGVVYITENKNKTVVIPCLGSISNLNVSLCARYPEKRFVPDGNRISWDSKKGFTIPSYMISYAGMVFCEAKINDESYQSIMYIVVVVGYRIYDVVLSPSHGIELSVGEKLVLNCTARTELNVGIDFNWEYPSSKHQHKKLVNRDLKTQSGSEMKKFLSTLTIDGVTRSDQGLYTCAASSGLMTKKNSTFVRVHEKPFVAFGSGMESLVEATVGERVRIPAKYLGYPPPEIKWYKNGIPLESNHTIKAGHVLTIMEVSERDTGNYTVILTNPISKEKQSHVVSLVVYVPPGPGDKTHTCPPCPAPELLGGPSVFLFPPKPKDTLMISRTPEVTCVVVDVSHEDPEVKFNWYVDGVEVHNAKTKPREEQYNSTYRVVSVLTVLHQDWLNGKEYKCKVSNKALPAPIEKTISKAKGQPREPQVYTLPPSRDELTKNQVSLTCLVKGFYPSDIAVEWESNGQPENNYKTTPPVLDSDGSFFLYSKLTVDKSRWQQGNVFSCSVMHEALHNHYTQKSLSLSPGK

SEQ ID NO: 36 - protein, 535 aa, Artificial sequence
  LFV-E recombinant receptor molecule
GLPSVSLDLPRLSIQKDILTIKANTTLQITCRGQRDLDWLWPNNQSGSEQRVEVTECSDGLFCKTLTIPKVIGNDTGAYKCFYRETDLASVIYVYVQDYRSPFIASVSDQHGVVYITENKNKTVVIPCLGSISNLNVSLCARYPEKRFVPDGNRISWDSKKGFTIPSYMISYAGMVFCEAKINDESYQSIMYIVVVVGYRIYDVVLSPSHGIELSVGEKLVLNCTARTELNVGIDFNWEYPSSKHQHKKLVNRDLKTQSGSEMKKFLSTLTIDGVTRSDQGLYTCAASSGLMTKKNSTFVRVHEKGPGDKTHTCPPCPAPELLGGPSVFLFPPKPKDTLMISRTPEVTCVVVDVSHEDPEVKFNWYVDGVEVHNAKTKPREEQYNSTYRVVSVLTVLHQDWLNGKEYKCKVSNKALPAPIEKTISKAKGQPREPQVYTLPPSRDELTKNQVSLTCLVKGFYPSDIAVEWESNGQPENNYKTTPPVLDSDGSFFLYSKLTVDKSRWQQGNVFSCSVMHEALHNHYTQKSLSLSPGK

SEQ ID NO: 37 - protein, 629 aa, Artificial sequence
  LFV-F recombinant receptor molecule
GLPSVSLDLPRLSIQKDILTIKANTTLQITCRGQRDLDWLWPNNQSGSEQRVEVTECSDGLFCKTLTIPKVIGNDTGAYKCFYRETDLASVIYVYVQDYRSPFIASVSDQHGVVYITENKNKTVVIPCLGSISNLNVSLCARYPEKRFVPDGNRISWDSKKGFTIPSYMISYAGMVFCEAKINDESYQSIMYIVVVVGYRIYDVVLSPSHGIELSVGEKLVLNCTARTELNVGIDFNWEYPSSKHQHKKLVNRDLKTQSGSEMKKFLSTLTIDGVTRSDQGLYTCAASSGLMTKKNSTFVRVHEKPFVAFGSGMESLVEATVGERVRIPAKYLGYPPPEIKWYKNGIPLESNHTIKAGHVLTIMEVSERDTGNYTVILTNPISKEKQSHVVSLVVYVPPGPGDKTHTCPPCPAPELLGGPSVFLFPPKPKDTLMISRTPEVTCVVVDVSHEDPEVKFNWYVDGVEVHNAKTKPREEQYNSTYRVVSVLTVLHQDWLNGKEYKCKVSNKALPAPIEKTISKAKGQPREPQVYTLPPSRDELTKNQVSLTCLVKGFYPSDIAVEWESNGQPENNYKTTPPVLDSDGSFFLYSKLTVDKSRWQQGNVFSCSVMHEALHNHYTQKSLSLSPGK

SEQ ID NO: 38 - protein, 435 aa, Artificial sequence
  LFV-G recombinant receptor molecule
SPFIASVSDQHGVVYITENKAKTVVIPCLGSISNLNVSLCARYPEKRFVPDGNRISWDSKKGFTIPSYMISYAGMVFCEAKINDESYQSIMYIVVVVGYRIYDVVLSPSHGIELSVGEKLVLNCTARTELNVGIDFNWEYPSSKHQHKKLVNRDLKTQSGSEMKKFLSTLTIDGVTRSDQGLYTCAASSGLMTKKNSTFVRVHEKGPGDKTHTCPPCPAPELLGGPSVFLFPPKPKDTLMISRTPEVTCVVVDVSHEDPEVKFNWYVDGVEVHNAKTKPREEQYNSTYRVVSVLTVLHQDWLNGKEYKCKVSNKALPAPIEKTISKAKGQPREPQVYTLPPSRDELTKNQVSLTCLVKGFYPSDIAVEWESNGQPENNYKTTPPVLDSDGSFFLYSKLTVDKSRWQQGNVFSCSVMHEALHNHYTQKSLSLSPGK

SEQ ID NO: 39 - protein, 435 aa, Artificial sequence
  LFV-H recombinant receptor molecule
SPFIASVSDQHGVVYITENKQKTVVIPCLGSISNLNVSLCARYPEKRFVPDGNRISWDSKKGFTIPSYMISYAGMVFCEAKINDESYQSIMYIVVVVGYRIYDVVLSPSHGIELSVGEKLVLNCTARTELNVGIDFNWEYPSSKHQHKKLVNRDLKTQSGSEMKKFLSTLTIDGVTRSDQGLYTCAASSGLMTKKNSTFVRVHEKGPGDKTHTCPPCPAPELLGGPSVFLFPPKPKDTLMISRTPEVTCVVVDVSHEDPEVKFNWYVDGVEVHNAKTKPREEQYNSTYRVVSVLTVLHQDWLNGKEYKCKVSNKALPAPIEKTISKAKGQPREPQVYTLPPSRDELTKNQVSLTCLVKGFYPSDIAVEWESNGQPENNYKTTPPVLDSDGSFFLYSKLTVDKSRWQQGNVFSCSVMHEALHNHYTQKSLSLSPGK

SEQ ID NO: 40 - protein, 435 aa, Artificial sequence
  LFV-I recombinant receptor molecule
SPFIASVSDQHGVVYITENKNKTVVIPCLGSISNLAVSLCARYPEKRFVPDGNRISWDSKKGFTIPSYMISYAGMVFCEAKINDESYQSIMYIVVVVGYRIYDVVLSPSHGIELSVGEKLVLNCTARTELNVGIDFNWEYPSSKHQHKKLVNRDLKTQSGSEMKKFLSTLTIDGVTRSDQGLYTCAASSGLMTKKNSTFVRVHEKGPGDKTHTCPPCPAPELLGGPSVFLFPPKPKDTLMISRTPEVTCVVVDVSHEDPEVKFNWYVDGVEVHNAKTKPREEQYNSTYRVVSVLTVLHQDWLNGKEYKCKVSNKALPAPIEKTISKAKGQPREPQVYTLPPSRDELTKNQVSLTCLVKGFYPSDIAVEWESNGQPENNYKTTPPVLDSDGSFFLYSKLTVDKSRWQQGNVFSCSVMHEALHNHYTQKSLSLSPGK

SEQ ID NO: 41 - protein, 435 aa, Artificial sequence
  LFV-J recombinant receptor molecule
SPFIASVSDQHGVVYITENKNKTVVIPCLGSISNLQVSLCARYPEKRFVPDGNRISWDSKKGFTIPSYMISYAGMVFCEAKINDESYQSIMYIVVVVGYRIYDVVLSPSHGIELSVGEKLVLNCTARTELNVGIDFNWEYPSSKHQHKKLVNRDLKTQSGSEMKKFLSTLTIDGVTRSDQGLYTCAASSGLMTKKNSTFVRVHEKGPGDKTHTCPPCPAPELLGGPSVFLFPPKPKDTLMISRTPEVTCVVVDVSHEDPEVKFNWYVDGVEVHNAKTKPREEQYNSTYRVVSVLTVLHQDWLNGKEYKCKVSNKALPAPIEKTISKAKGQPREPQVYTLPPSRDELTKNQVSLTCLVKGFYPSDIAVEWESNGQPENNYKTTPPVLDSDGSFFLYSKLTVDKSRWQQGNVFSCSVMHEALHNHYTQKSLSLSPGK

SEQ ID NO: 42 - protein, 435 aa, Artificial sequence
  LFV-K recombinant receptor molecule
SPFIASVSDQHGVVYITENKNKTVVIPCLGSISNLNVSLCARYPEKRFVPDGNRISWDSKKGFTIPSYMISYAGMVFCEAKINDESYQSIMYIVVVVGYRIYDVVLSPSHGIELSVGEKLVLQCTARTELNVGIDFNWEYPSSKHQHKKLVNRDLKTQSGSEMKKFLSTLTIDGVTRSDQGLYTCAASSGLMTKKNSTFVRVHEKGPGDKTHTCPPCPAPELLGGPSVFLFPPKPKDTLMISRTPEVTCVVVDVSHEDPEVKFNWYVDGVEVHNAKTKPREEQYNSTYRVVSVLTVLHQDWLNGKEYKCKVSNKALPAPIEKTISKAKGQPREPQVYTLPPSRDELTKNQVSLTCLVKGFYPSDIAVEWESNGQPENNYKTTPPVLDSDGSFFLYSKLTVDKSRWQQGNVFSCSVMHEALHNHYTQKSLSLSPGK

SEQ ID NO: 43 - protein, 435 aa, Artificial sequence
  LFV-L recombinant receptor molecule
SPFIASVSDQHGVVYITENKNKTVVIPCLGSISNLNVSLCARYPEKRFVPDGNRISWDSKKGFTIPSYMISYAGMVFCEAKINDESYQSIMYIVVVVGYRIYDVVLSPSHGIELSVGEKLVLNCTARTELNVGIDFNWEYPSSKHQHKKLVNRDLKTQSGSEMKKFLSTLTIDGVTRSDQGLYTCAASSGLMTKKQSTFVRVHEKGPGDKTHTCPPCPAPELLGGPSVFLFPPKPKDTLMISRTPEVTCVVVDVSHEDPEVKFNWYVDGVEVHNAKTKPREEQYNSTYRVVSVLTVLHQDWLNGKEYKCKVSNKALPAPIEKTISKAKGQPREPQVYTLPPSRDELTKNQVSLTCLVKGFYPSDIAVEWESNGQPENNYKTTPPVLDSDGSFFLYSKLTVDKSRWQQGNVFSCSVMHEALHNHYTQKSLSLSPGK

SEQ ID NO: 44 - protein, 541 aa, Artificial sequence
  LFV-M recombinant receptor molecule
GRPFVEMYSEIPEIIHMTEGRELVIPCRVTSPNITVTLKKFPLDTLIPDGKRIIWDSRKGFIISNATYKEIGLLTCEATVNGHLYKTNYLTHRQTNTIIGGGGSGGSPFIASVSDQHGVVYITENKNKTVVIPCLGSISNLNVSLCARYPEKRFVPDGNRISWDSKKGFTIPSYMISYAGMVFCEAKINDESYQSIMYIVVVVGYRIYDVVLSPSHGIELSVGEKLVLNCTARTELNVGIDFNWEYPSSKHQHKKLVNRDLKTQSGSEMKKFLSTLTIDGVTRSDQGLYTCAASSGLMTKKNSTFVRVHEKGPGDKTHTCPPCPAPELLGGPSVFLFPPKPKDTLMISRTPEVTCVVVDVSHEDPEVKFNWYVDGVEVHNAKTKPREEQYNSTYRVVSVLTVLHQDWLNGKEYKCKVSNKALPAPIEKTISKAKGQPREPQVYTLPPSRDELTKNQVSLTCLVKGFYPSDIAVEWESNGQPENNYKTTPPVLDSDGSFFLYSKLTVDKSRWQQGNVFSCSVMHEALHNHYTQKSLSLSPGK

SEQ ID NO: 45 - protein, 539 aa, Artificial sequence
  LFV-N recombinant receptor molecule
SPFIASVSDQHGVVYITENKNKTVVIPCLGSISNLNVSLCARYPEKRFVPDGNRISWDSKKGFTIPSYMISYAGMVFCEAKINDESYQSIMYIVVVVGYRIYDVVLSPSHGIELSVGEKLVLNCTARTELNVGIDFNWEYPSSKHQHKKLVNRDLKTQSGSEMKKFLSTLTIDGVTRSDQGLYTCAASSGLMTKKNSTFVRVHEKGGGGSGRPFVEMYSEIPEIIHMTEGRELVIPCRVTSPNITVTLKKFPLDTLIPDGKRIIWDSRKGFIISNATYKEIGLLTCEATVNGHLYKTNYLTHRQTNTIIGPGDKTHTCPPCPAPELLGGPSVFLFPPKPKDTLMISRTPEVTCVVVDVSHEDPEVKFNWYVDGVEVHNAKTKPREEQYNSTYRVVSVLTVLHQDWLNGKEYKCKVSNKALPAPIEKTISKAKGQPREPQVYTLPPSRDELTKNQVSLTCLVKGFYPSDIAVEWESNGQPENNYKTTPPVLDSDGSFFLYSKLTVDKSRWQQGNVFSCSVMHEALHNHYTQKSLSLSPGK

SEQ ID NO: 46 - protein, 652 aa, Artificial sequence
  LFV-O recombinant receptor molecule
SPFIASVSDQHGVVYITENKNKTVVIPCLGSISNLNVSLCARYPEKRFVPDGNRISWDSKKGFTIPSYMISYAGMVFCEAKINDESYQSIMYIVVVVGYRIYDVVLSPSHGIELSVGEKLVLNCTARTELNVGIDFNWEYPSSKHQHKKLVNRDLKTQSGSEMKKFLSTLTIDGVTRSDQGLYTCAASSGLMTKKNSTFVRVHEKGPGDKTHTCPPCPAPELLGGPSVFLFPPKPKDTLMISRTPEVTCVVVDVSHEDPEVKFNWYVDGVEVHNAKTKPREEQYNSTYRVVSVLTVLHQDWLNGKEYKCKVSNKALPAPIEKTISKAKGQPREPQVYTLPPSRDELTKNQVSLTCLVKGFYPSDIAVEWESNGQPENNYKTTPPVLDSDGSFFLYSKLTVDKSRWQQGNVFSCSVMHEALHNHYTQKSLSLSPGAGGGGSGGGGSGGGGSGRPFVEMYSEIPEIIHMTEGRELVIPCRVTSPNITVTLKKFPLDTLIPDGKRIIWDSRKGFIISNATYKEIGLLTCEATVNGHLYKTNYLTHRQTNTIIDVVLSPSHGIELSVGEKLVLNCTARTELNVGIDFNWEYPSSKHQHKKLVNRDLKTQSGSEMKKFLSTLTIDGVTRSDQGLYTCAASSGLMTKKNSTFVRVHEK

SEQ ID NO: 47 - protein, 441 aa, Artificial sequence
  LFV-P recombinant receptor molecule
YVQDYRSPFIASVSDQHGVVYITENKNKTVVIPCLGSISNLNVSLCARYPEKRFVPDGNRISWDSKKGFTIPSYMISYAGMVFCEAKINDESYQSIMYIVVVVGYRIYDVVLSPSHGIELSVGEKLVLQCTARTELNVGIDFNWEYPSSKHQHKKLVNRDLKTQSGSEMKKFLSTLTIDGVTRSDQGLYTCAASSGLMTKKNSTFVRVHEKGPGDKTHTCPPCPAPELLGGPSVFLFPPKPKDTLMISRTPEVTCVVVDVSHEDPEVKFNWYVDGVEVHNAKTKPREEQYNSTYRVVSVLTVLHQDWLNGKEYKCKVSNKALPAPIEKTISKAKGQPREPQVYTLPPSRDELTKNQVSLTCLVKGFYPSDIAVEWESNGQPENNYKTTPPVLDSDGSFFLYSKLTVDKSRWQQGNVFSCSVMHEALHNHYTQKSLSLSPGK

SEQ ID NO: 48 - protein, 545 aa, Artificial sequence
  LFV-Q recombinant receptor molecule
YVQDYRSPFIASVSDQHGVVYITENKNKTVVIPCLGSISNLNVSLCARYPEKRFVPDGNRISWDSKKGFTIPSYMISYAGMVFCEAKINDESYQSIMYIVVVVGYRIYDVVLSPSHGIELSVGEKLVLQCTARTELNVGIDFNWEYPSSKHQHKKLVNRDLKTQSGSEMKKFLSTLTIDGVTRSDQGLYTCAASSGLMTKKNSTFVRVHEKGGGGSGRPFVEMYSEIPEIIHMTEGRELVIPCRVTSPNITVTLKKFPLDTLIPDGKRIIWDSRKGFIISNATYKEIGLLTCEATVNGHLYKTNYLTHRQTNTIIGPGDKTHTCPPCPAPELLGGPSVFLFPPKPKDTLMISRTPEVTCVVVDVSHEDPEVKFNWYVDGVEVHNAKTKPREEQYNSTYRVVSVLTVLHQDWLNGKEYKCKVSNKALPAPIEKTISKAKGQPREPQVYTLPPSRDELTKNQVSLTCLVKGFYPSDIAVEWESNGQPENNYKTTPPVLDSDGSFFLYSKLTVDKSRWQQGNVFSCSVMHEALHNHYTQKSLSLSPGK

SEQ ID NO: 49 - protein, 541 aa, Artificial sequence
  LFV-R recombinant receptor molecule
GRPFVEMYSEIPEIIHMTEGRELVIPCRVTSPNITVTLKKFPLDTLIPDGKRIIWDSRKGFIISNATYKEIGLLTCEATVNGHLYKTNYLTHRQTNTIIGGGGSGGSPFIASVSDQHGVVYITENKNKTVVIPCLGSISNLNVSLCARYPEKRFVPDGNRISWDSKKGFTIPSYMISYAGMVFCEAKINDESYQSIMYIVVVVGYRIYDVVLSPSHGIELSVGEKLVLQCTARTELNVGIDFNWEYPSSKHQHKKLVNRDLKTQSGSEMKKFLSTLTIDGVTRSDQGLYTCAASSGLMTKKNSTFVRVHEKGPGDKTHTCPPCPAPELLGGPSVFLFPPKPKDTLMISRTPEVTCVVVDVSHEDPEVKFNWYVDGVEVHNAKTKPREEQYNSTYRVVSVLTVLHQDWLNGKEYKCKVSNKALPAPIEKTISKAKGQPREPQVYTLPPSRDELTKNQVSLTCLVKGFYPSDIAVEWESNGQPENNYKTTPPVLDSDGSFFLYSKLTVDKSRWQQGNVFSCSVMHEALHNHYTQKSLSLSPGK

SEQ ID NO: 50 - protein, 545 aa, Artificial sequence
  LFV-S recombinant receptor molecule
YVQDYRSPFIASVSDQHGVVYITENKNKTVVIPCLGSISNLNVSLCARYPEKRFVPDGNRISWDSKKGFTIPSYMISYAGMVFCEAKINDESYQSIMYIVVVVGYRIYDVVLSPSHGIELSVGEKLVLNCTARTELNVGIDFNWEYPSSKHQHKKLVNRDLKTQSGSEMKKFLSTLTIDGVTRSDQGLYTCAASSGLMTKKNSTFVRVHEKGGGGSGRPFVEMYSEIPEIIHMTEGRELVIPCRVTSPNITVTLKKFPLDTLIPDGKRIIWDSRKGFIISNATYKEIGLLTCEATVNGHLYKTNYLTHRQTNTIIGPGDKTHTCPPCPAPELLGGPSVFLFPPKPKDTLMISRTPEVTCVVVDVSHEDPEVKFNWYVDGVEVHNAKTKPREEQYNSTYRVVSVLTVLHQDWLNGKEYKCKVSNKALPAPIEKTISKAKGQPREPQVYTLPPSRDELTKNQVSLTCLVKGFYPSDIAVEWESNGQPENNYKTTPPVLDSDGSFFLYSKLTVDKSRWQQGNVFSCSVMHEALHNHYTQKSLSLSPGK

SEQ ID NO: 51 - protein, 539 aa, Artificial sequence
  LFV-001 recombinant receptor molecule
YSMTPPTLNITEESHVIDTGDSLSISCRGQHPLEWAWPGAQEAPATGDKDSEDTGVVRDCEGTDARPYCKVLLLHEVHANDTGSYVCYYKYIKARIEGTTAASSYVFVRDFEQPFINKPDTLLVNRKDAMWVPCLVSIPGLNVTLRSQSSVLWPDGQEVVWDDRRGMLVSTPLLHDALYLQCETTWGDQDFLSNPFLVHITGYRIYDVVLSPSHGIELSVGEKLVLNCTARTELNVGIDFNWEYPSSKHQHKKLVNRDLKTQSGSEMKKFLSTLTIDGVTRSDQGLYTCAASSGLMTKKNSTFVRVHEKGPGDKTHTCPPCPAPELLGGPSVFLFPPKPKDTLMISRTPEVTCVVVDVSHEDPEVKFNWYVDGVEVHNAKTKPREEQYNSTYRVVSVLTVLHQDWLNGKEYKCKVSNKALPAPIEKTISKAKGQPREPQVYTLPPSRDELTKNQVSLTCLVKGFYPSDIAVEWESNGQPENNYKTTPPVLDSDGSFFLYSKLTVDKSRWQQGNVFSCSVMHEALHNHYTQKSLSLSPGK

SEQ ID NO: 52 - protein, 539 aa, Artificial sequence
  LFV-010 recombinant receptor molecule
YSMTPPTLNITEESHVIDTGDSLSISCRGQHPLEWAWPGAQEAPATGDKDSEDTGVVRDCEGTDARPYCKVLLLHEVHAQDTGSYVCYYKYIKARIEGTTAASSYVFVRDFEQPFINKPDTLLVNRKDAMWVPCLVSIPGLNVTLRSQSSVLWPDGQEVVWDDRRGMLVSTPLLHDALYLQCETTWGDQDFLSNPFLVHITGNELYDVVLSPSHGIELSVGEKLVLNCTARTELNVGIDFNWEYPSSKHQHKKLVNRDLKTQSGSEMKKFLSTLTIDGVTRSDQGLYTCAASSGLMTKKNSTFVRVHEKGPGDKTHTCPPCPAPELLGGPSVFLFPPKPKDTLMISRTPEVTCVVVDVSHEDPEVKFNWYVDGVEVHNAKTKPREEQYNSTYRVVSVLTVLHQDWLNGKEYKCKVSNKALPAPIEKTISKAKGQPREPQVYTLPPSRDELTKNQVSLTCLVKGFYPSDIAVEWESNGQPENNYKTTPPVLDSDGSFFLYSKLTVDKSRWQQGNVFSCSVMHEALHNHYTQKSLSLSPGK

SEQ ID NO: 53 - protein, 538 aa, Artificial sequence
  LFV-002 recombinant receptor molecule
YSMTPPTLNITEESHVIDTGDSLSISCRGQHPLEWAWPGAQEAPATGDKDSEDTGVVRDCEGTDARPYCKVLLLHEVHANDTGSYVCYYKYIKARIEGTTAASSYVFVRDFEQPFINKPDTLLVNRKDAMWVPCLVSIPGLNVTLRSQSSVLWPDGQEVVWDDRRGMLVSTPLLHDALYLQCETTWGDQDFLSNPFLVHIGYRIYDVVLSPSHGIELSVGEKLVLNCTARTELNVGIDFNWEYPSSKHQHKKLVNRDLKTQSGSEMKKFLSTLTIDGVTRSDQGLYTCAASSGLMTKKNSTFVRVHEKGPGDKTHTCPPCPAPELLGGPSVFLFPPKPKDTLMISRTPEVTCVVVDVSHEDPEVKFNWYVDGVEVHNAKTKPREEQYNSTYRVVSVLTVLHQDWLNGKEYKCKVSNKALPAPIEKTISKAKGQPREPQVYTLPPSRDELTKNQVSLTCLVKGFYPSDIAVEWESNGQPENNYKTTPPVLDSDGSFFLYSKLTVDKSRWQQGNVFSCSVMHEALHNHYTQKSLSLSPGK

SEQ ID NO: 54 - protein, 539 aa, Artificial sequence
  LFV-003 recombinant receptor molecule
YSMTPPTLNITEESHVIDTGDSLSISCRGQHPLEWAWPGAQEAPATGDKDSEDTGVVRDCEGTDARPYCKVLLLHEVHANDTGSYVCYYKYIKARIEGTTAASSYVFVRDFEQPFINKPDTLLVNRKDAMWVPCLVSIPGLNVTLRSQSSVLWPDGQEVVWDDRRGMLVSTPLLHDALYLQCETTWGDQDFLSNPFLVHIGGYRIYDVVLSPSHGIELSVGEKLVLNCTARTELNVGIDFNWEYPSSKHQHKKLVNRDLKTQSGSEMKKFLSTLTIDGVTRSDQGLYTCAASSGLMTKKNSTFVRVHEKGPGDKTHTCPPCPAPELLGGPSVFLFPPKPKDTLMISRTPEVTCVVVDVSHEDPEVKFNWYVDGVEVHNAKTKPREEQYNSTYRVVSVLTVLHQDWLNGKEYKCKVSNKALPAPIEKTISKAKGQPREPQVYTLPPSRDELTKNQVSLTCLVKGFYPSDIAVEWESNGQPENNYKTTPPVLDSDGSFFLYSKLTVDKSRWQQGNVFSCSVMHEALHNHYTQKSLSLSPGK

SEQ ID NO: 55 - protein, 539 aa, Artificial sequence
  LFV-004 recombinant receptor molecule
YSMTPPTLNITEESHVIDTGDSLSISCRGQHPLEWAWPGAQEAPATGDKDSEDTGVVRDCEGTDARPYCKVLLLHEVHANDTGSYVCYYKYIKARIEGTTAASSYVFVRDFEQPFINKPDTLLVNRKDAMWVPCLVSIPGLNVTLRSQSSVLWPDGQEVVWDDRRGMLVSTPLLHDALYLQCETTWGDQDFLSNPFIVHVTGYRIYDVVLSPSHGIELSVGEKLVLNCTARTELNVGIDFNWEYPSSKHQHKKLVNRDLKTQSGSEMKKFLSTLTIDGVTRSDQGLYTCAASSGLMTKKNSTFVRVHEKGPGDKTHTCPPCPAPELLGGPSVFLFPPKPKDTLMISRTPEVTCVVVDVSHEDPEVKFNWYVDGVEVHNAKTKPREEQYNSTYRVVSVLTVLHQDWLNGKEYKCKVSNKALPAPIEKTISKAKGQPREPQVYTLPPSRDELTKNQVSLTCLVKGFYPSDIAVEWESNGQPENNYKTTPPVLDSDGSFFLYSKLTVDKSRWQQGNVFSCSVMHEALHNHYTQKSLSLSPGK

SEQ ID NO: 56 - protein, 539 aa, Artificial sequence
  LFV-005 recombinant receptor molecule
YSMTPPTLNITEESHVIDTGDSLSISCRGQHPLEWAWPGAQEAPATGDKDSEDTGVVRDCEGTDARPYCKVLLLHEVHANDTGSYVCYYKYIKARIEGTTAASSYVFVRDFEQPFINKPDTLLVNRKDAMWVPCLVSIPGLNVTLRSQSSVLWPDGQEVVWDDRRGMLVSTPLLHDALYLQCETTWGDQDFLSNPFIVVVVGYRIYDVVLSPSHGIELSVGEKLVLNCTARTELNVGIDFNWEYPSSKHQHKKLVNRDLKTQSGSEMKKFLSTLTIDGVTRSDQGLYTCAASSGLMTKKNSTFVRVHEKGPGDKTHTCPPCPAPELLGGPSVFLFPPKPKDTLMISRTPEVTCVVVDVSHEDPEVKFNWYVDGVEVHNAKTKPREEQYNSTYRVVSVLTVLHQDWLNGKEYKCKVSNKALPAPIEKTISKAKGQPREPQVYTLPPSRDELTKNQVSLTCLVKGFYPSDIAVEWESNGQPENNYKTTPPVLDSDGSFFLYSKLTVDKSRWQQGNVFSCSVMHEALHNHYTQKSLSLSPGK

SEQ ID NO: 57 - protein, 539 aa, Artificial sequence
  LFV-006 recombinant receptor molecule
YSMTPPTLNITEESHVIDTGDSLSISCRGQHPLEWAWPGAQEAPATGDKDSEDTGVVRDCEGTDARPYCKVLLLHEVHANDTGSYVCYYKYIKARIEGTTAASSYVFVRDFEQPFINKPDTLLVNRKDAMWVPCLVSIPGLNVTLRSQSSVLWPDGQEVVWDDRRGMLVSTPLLHDALYLQCETTWGDQDFLSNMYIVVVVGYRIYDVVLSPSHGIELSVGEKLVLNCTARTELNVGIDFNWEYPSSKHQHKKLVNRDLKTQSGSEMKKFLSTLTIDGVTRSDQGLYTCAASSGLMTKKNSTFVRVHEKGPGDKTHTCPPCPAPELLGGPSVFLFPPKPKDTLMISRTPEVTCVVVDVSHEDPEVKFNWYVDGVEVHNAKTKPREEQYNSTYRVVSVLTVLHQDWLNGKEYKCKVSNKALPAPIEKTISKAKGQPREPQVYTLPPSRDELTKNQVSLTCLVKGFYPSDIAVEWESNGQPENNYKTTPPVLDSDGSFFLYSKLTVDKSRWQQGNVFSCSVMHEALHNHYTQKSLSLSPGK

SEQ ID NO: 58 - protein, 539 aa, Artificial sequence
  LFV-007 recombinant receptor molecule
YSMTPPTLNITEESHVIDTGDSLSISCRGQHPLEWAWPGAQEAPATGDKDSEDTGVVRDCEGTDARPYCKVLLLHEVHANDTGSYVCYYKYIKARIEGTTAASSYVFVRDFEQPFINKPDTLLVNRKDAMWVPCLVSIPGLNVTLRSQSSVLWPDGQEVVWDDRRGMLVSTPLLHDALYLQCETTWGDQDFLSIMYIVVVVGYRIYDVVLSPSHGIELSVGEKLVLNCTARTELNVGIDFNWEYPSSKHQHKKLVNRDLKTQSGSEMKKFLSTLTIDGVTRSDQGLYTCAASSGLMTKKNSTFVRVHEKGPGDKTHTCPPCPAPELLGGPSVFLFPPKPKDTLMISRTPEVTCVVVDVSHEDPEVKFNWYVDGVEVHNAKTKPREEQYNSTYRVVSVLTVLHQDWLNGKEYKCKVSNKALPAPIEKTISKAKGQPREPQVYTLPPSRDELTKNQVSLTCLVKGFYPSDIAVEWESNGQPENNYKTTPPVLDSDGSFFLYSKLTVDKSRWQQGNVFSCSVMHEALHNHYTQKSLSLSPGK

SEQ ID NO: 59 - protein, 539 aa, Artificial sequence
  LFV-008 recombinant receptor molecule
YSMTPPTLNITEESHVIDTGDSLSISCRGQHPLEWAWPGAQEAPATGDKDSEDTGVVRDCEGTDARPYCKVLLLHEVHANDTGSYVCYYKYIKARIEGTTAASSYVFVRDFEQPFINKPDTLLVNRKDAMWVPCLVSIPGLNVTLRSQSSVLWPDGQEVVWDDRRGMLVSTPLLHDALYLQCETTWGDQDFLSAMYIVVVVGYRIYDVVLSPSHGIELSVGEKLVLNCTARTELNVGIDFNWEYPSSKHQHKKLVNRDLKTQSGSEMKKFLSTLTIDGVTRSDQGLYTCAASSGLMTKKNSTFVRVHEKGPGDKTHTCPPCPAPELLGGPSVFLFPPKPKDTLMISRTPEVTCVVVDVSHEDPEVKFNWYVDGVEVHNAKTKPREEQYNSTYRVVSVLTVLHQDWLNGKEYKCKVSNKALPAPIEKTISKAKGQPREPQVYTLPPSRDELTKNQVSLTCLVKGFYPSDIAVEWESNGQPENNYKTTPPVLDSDGSFFLYSKLTVDKSRWQQGNVFSCSVMHEALHNHYTQKSLSLSPGK